European Patent Application EP 4 321 630 A1, published February 14, 2024. Title: Method for parallel, rapid and sensitive detection of DNA double strand breaks. Applicant: Insitute of Molecular Biology gGmbH (IMB). Application EP 22189451, filed August 9, 2022. The sequence listing filed with the application follows.

SEQUENCE LISTING (77 sequences)

SEQ ID NO: 1 - DNA, 14 bp, synthetic construct
  source 1..14: mol_type = other DNA
tcgtcggcagcgtc

SEQ ID NO: 2 - DNA, 33 bp, synthetic construct
  source 1..33: mol_type = other DNA
tcgtcggcagcgtcagatgtgtataagagacag

SEQ ID NO: 3 - DNA, 66 bp, synthetic construct
  source 1..66: mol_type = other DNA
  unsure 50..57: note = Unique Molecular Identifier (UMI)
cgattgaggccgggtctcgtcggcagcgtcagatgtgtataagagacagnnnnnnnnctcacacgt

SEQ ID NO: 4 - DNA, 67 bp, synthetic construct
  source 1..67: mol_type = other DNA
  unsure 9..16: note = Unique Molecular Identifier (UMI)
cgtgtgagnnnnnnnnctgtctcttatacacatctgacgctgccgacgagacccggcctcaatcgaa

SEQ ID NO: 5 - DNA, 19 bp, synthetic construct
  source 1..19: mol_type = other DNA
ctgtctcttatacacatct

SEQ ID NO: 6 - DNA, 15 bp, synthetic construct
  source 1..15: mol_type = other DNA
gtctcgtgggctcgg

SEQ ID NO: 7 - DNA, 34 bp, synthetic construct
  source 1..34: mol_type = other DNA
gtctcgtgggctcggagatgtgtataagagacag

SEQ ID NO: 8 - DNA, 51 bp, synthetic construct
  source 1..51: mol_type = other DNA
  unsure 30..37: note = i5 index sequence
aatgatacggcgaccaccgagatctacacnnnnnnnntcgtcggcagcgtc

SEQ ID NO: 9 - DNA, 47 bp, synthetic construct
  source 1..47: mol_type = other DNA
  unsure 25..32: note = i7 index sequence
caagcagaagacggcatacgagatnnnnnnnngtctcgtgggctcgg

SEQ ID NO: 10 - DNA, 66 bp, synthetic construct
  source 1..66: mol_type = other DNA
  unsure 50..57: note = Unique Molecular Identifier (UMI)
  unsure 58..65: note = Barcode Region
cgattgaggccgggtctcgtcggcagcgtcagatgtgtataagagacagnnnnnnnnnnnnnnnnt

SEQ ID NO: 11 - DNA, 67 bp, synthetic construct
  source 1..67: mol_type = other DNA
  unsure 1..8: note = Barcode Region
  unsure 9..16: note = Unique Molecular Identifier (UMI)
nnnnnnnnnnnnnnnnctgtctcttatacacatctgacgctgccgacgagacccggcctcaatcgaa

SEQ ID NO: 12 - DNA, 27 bp, Homo sapiens
  source 1..27: mol_type = genomic DNA
cgttccaagaactataggtccgcagac

SEQ ID NO: 13 - DNA, 35 bp, Homo sapiens
  source 1..35: mol_type = genomic DNA
aggaggaagtgactggacctcagaagagtgcgacc

SEQ ID NO: 14 - DNA, 21 bp, Homo sapiens
  source 1..21: mol_type = genomic DNA
caaaccacgctagcgcactct

SEQ ID NO: 15 - DNA, 23 bp, Homo sapiens
  source 1..23: mol_type = genomic DNA
agatggaaagtccaggacggaac

SEQ ID NO: 16 - DNA, 22 bp, Homo sapiens
  source 1..22: mol_type = genomic DNA
ttgttcggactgagtcccaaac

SEQ ID NO: 17 - DNA, 40 bp, Homo sapiens
  source 1..40: mol_type = genomic DNA
gtctcgacgaggactcaagtatacaggaatccgttgacag

SEQ ID NO: 18 - DNA, 35 bp, Homo sapiens
  source 1..35: mol_type = genomic DNA
cgacgcagtcgagaaggagaggatcctccctgggg

SEQ ID NO: 19 - DNA, 27 bp, Homo sapiens
  source 1..27: mol_type = genomic DNA
cccgaccccctccaccccgcctccggg

SEQ ID NO: 20 - DNA, 27 bp, Homo sapiens
  source 1..27: mol_type = genomic DNA
gggctgggggaggtggggcggaggccc

SEQ ID NO: 21 - DNA, 20 bp, Homo sapiens
  source 1..20: mol_type = genomic DNA
cccgaccccctccaccccgc

SEQ ID NO: 22 - DNA, 20 bp, Homo sapiens
  source 1..20: mol_type = genomic DNA
gggctgggggaggtggggcg

SEQ ID NO: 23 - DNA, 27 bp, Homo sapiens
  source 1..27: mol_type = genomic DNA
cccgaccccctccaccccgcctccggg

SEQ ID NO: 24 - DNA, 27 bp, Homo sapiens
  source 1..27: mol_type = genomic DNA
gggctgggggaggtggggcggaggccc

SEQ ID NO: 25 - DNA, 19 bp, Homo sapiens
  source 1..19: mol_type = other DNA
cccgaccccctccaccccg

SEQ ID NO: 26 - DNA, 20 bp, Homo sapiens
  source 1..20: mol_type = genomic DNA
gggctgggggaggtggggcg

SEQ ID NO: 27 - DNA, 20 bp, synthetic construct
  source 1..20: mol_type = other DNA
cccgaccccctccaccccgc

SEQ ID NO: 28 - DNA, 35 bp, Homo sapiens
  source 1..35: mol_type = genomic DNA
gctgcagaaacagcaagcccaggaactgagcctcc

SEQ ID NO: 29 - DNA, 40 bp, Homo sapiens
  source 1..40: mol_type = genomic DNA
tcaagtcggatggtctccaccccacccccctgactaagta

SEQ ID NO: 30 - RNA, 100 nt, synthetic construct
  source 1..100: mol_type = other RNA
  modified_base 1..3: mod_base = OTHER; note = 2-O-methyl phosphorothioate nucleotides
  modified_base 97..99: mod_base = OTHER; note = 2-O-methyl phosphorothioate nucleotides
gtcaccaatcctgtccctaggttttagagctagaaatagcaagttaaaataaggctagtccgttatcaacttgaaaaagtggcaccgagtcggtgctttt

SEQ ID NO: 31 - RNA, 100 nt, synthetic construct
  source 1..100: mol_type = other RNA
  modified_base 1..3: mod_base = OTHER; note = 2-O-methyl phosphorothioate nucleotides
  modified_base 97..99: mod_base = OTHER; note = 2-O-methyl phosphorothioate nucleotides
ggcagaaaccctggtggtcggttttagagctagaaatagcaagttaaaataaggctagtccgttatcaacttgaaaaagtggcaccgagtcggtgctttt

SEQ ID NO: 32 - RNA, 100 nt, synthetic construct
  source 1..100: mol_type = other RNA
  modified_base 1..3: mod_base = OTHER; note = 2-O-methyl phosphorothioate nucleotides
  modified_base 97..99: mod_base = OTHER; note = 2-O-methyl phosphorothioate nucleotides
gcacgtggcccagcctgctggttttagagctagaaatagcaagttaaaataaggctagtccgttatcaacttgaaaaagtggcaccgagtcggtgctttt

SEQ ID NO: 33 - RNA, 100 nt, synthetic construct
  source 1..100: mol_type = other RNA
  modified_base 1..3: mod_base = OTHER; note = 2-O-methyl phosphorothioate nucleotides
  modified_base 97..99: mod_base = OTHER; note = 2-O-methyl phosphorothioate nucleotides
gagggctcaccagaggtagggttttagagctagaaatagcaagttaaaataaggctagtccgttatcaacttgaaaaagtggcaccgagtcggtgctttt

SEQ ID NO: 34 - RNA, 100 nt, synthetic construct
  source 1..100: mol_type = other RNA
  modified_base 1..3: mod_base = OTHER; note = 2-O-methyl phosphorothioate nucleotides
  modified_base 97..99: mod_base = OTHER; note = 2-O-methyl phosphorothioate nucleotides
ggcgccctggccagtcgtctgttttagagctagaaatagcaagttaaaataaggctagtccgttatcaacttgaaaaagtggcaccgagtcggtgctttt

SEQ ID NO: 35 - RNA, 100 nt, synthetic construct
  source 1..100: mol_type = other RNA
  modified_base 1..3: mod_base = OTHER; note = 2-O-methyl phosphorothioate nucleotides
  modified_base 97..99: mod_base = OTHER; note = 2-O-methyl phosphorothioate nucleotides
gtcagggttctggatatctggttttagagctagaaatagcaagttaaaataaggctagtccgttatcaacttgaaaaagtggcaccgagtcggtgctttt

SEQ ID NO: 36 - RNA, 100 nt, synthetic construct
  source 1..100: mol_type = other RNA
  modified_base 1..3: mod_base = OTHER; note = 2-O-methyl phosphorothioate nucleotides
  modified_base 97..99: mod_base = OTHER; note = 2-O-methyl phosphorothioate nucleotides
gggaacccagcgagtgaagagttttagagctagaaatagcaagttaaaataaggctagtccgttatcaacttgaaaaagtggcaccgagtcggtgctttt

SEQ ID NO: 37 - RNA, 100 nt, synthetic construct
  source 1..100: mol_type = other RNA
  modified_base 1..3: mod_base = OTHER; note = 2-O-methyl phosphorothioate nucleotides
  modified_base 97..99: mod_base = OTHER; note = 2-O-methyl phosphorothioate nucleotides
gatttcctcctcgaccaccagttttagagctagaaatagcaagttaaaataaggctagtccgttatcaacttgaaaaagtggcaccgagtcggtgctttt

SEQ ID NO: 38 - RNA, 100 nt, synthetic construct
  source 1..100: mol_type = other RNA
  modified_base 1..3: mod_base = OTHER; note = 2-O-methyl phosphorothioate nucleotides
  modified_base 97..99: mod_base = OTHER; note = 2-O-methyl phosphorothioate nucleotides
gaggttcacttgatttccacgttttagagctagaaatagcaagttaaaataaggctagtccgttatcaacttgaaaaagtggcaccgagtcggtgctttt

SEQ ID NO: 39 - RNA, 100 nt, synthetic construct
  source 1..100: mol_type = other RNA
  modified_base 1..3: mod_base = OTHER; note = 2-O-methyl phosphorothioate nucleotides
  modified_base 97..99: mod_base = OTHER; note = 2-O-methyl phosphorothioate nucleotides
gctgaccccgctgggcaggcgttttagagctagaaatagcaagttaaaataaggctagtccgttatcaacttgaaaaagtggcaccgagtcggtgctttt

SEQ ID NO: 40 - RNA, 100 nt, synthetic construct
  source 1..100: mol_type = other RNA
  modified_base 1..3: mod_base = OTHER; note = 2-O-methyl phosphorothioate nucleotides
  modified_base 97..99: mod_base = OTHER; note = 2-O-methyl phosphorothioate nucleotides
ggagaaggtgggggggttccgttttagagctagaaatagcaagttaaaataaggctagtccgttatcaacttgaaaaagtggcaccgagtcggtgctttt

SEQ ID NO: 41 - RNA, 100 nt, synthetic construct
  source 1..100: mol_type = other RNA
  modified_base 1..3: mod_base = OTHER; note = 2-O-methyl phosphorothioate nucleotides
  modified_base 97..99: mod_base = OTHER; note = 2-O-methyl phosphorothioate nucleotides
gctggtacacggcagggtcagttttagagctagaaatagcaagttaaaataaggctagtccgttatcaacttgaaaaagtggcaccgagtcggtgctttt

SEQ ID NO: 42 - RNA, 100 nt, synthetic construct
  source 1..100: mol_type = other RNA
  modified_base 1..3: mod_base = OTHER; note = 2-O-methyl phosphorothioate nucleotides
  modified_base 97..99: mod_base = OTHER; note = 2-O-methyl phosphorothioate nucleotides
ggtgagggaggagagatgccgttttagagctagaaatagcaagttaaaataaggctagtccgttatcaacttgaaaaagtggcaccgagtcggtgctttt

SEQ ID NO: 43 - RNA, 100 nt, synthetic construct
  source 1..100: mol_type = other RNA
  modified_base 1..3: mod_base = OTHER; note = 2-O-methyl phosphorothioate nucleotides
  modified_base 97..99: mod_base = OTHER; note = 2-O-methyl phosphorothioate nucleotides
ggatttcctcctcgaccaccgttttagagctagaaatagcaagttaaaataaggctagtccgttatcaacttgaaaaagtggcaccgagtcggtgctttt

SEQ ID NO: 44 - RNA, 100 nt, synthetic construct
  source 1..100: mol_type = other RNA
  modified_base 1..3: mod_base = OTHER; note = 2-O-methyl phosphorothioate nucleotides
  modified_base 97..99: mod_base = OTHER; note = 2-O-methyl phosphorothioate nucleotides
ggccagtaccacagcaggctgttttagagctagaaatagcaagttaaaataaggctagtccgttatcaacttgaaaaagtggcaccgagtcggtgctttt

SEQ ID NO: 45 - RNA, 100 nt, synthetic construct
  source 1..100: mol_type = other RNA
  modified_base 1..3: mod_base = OTHER; note = 2-O-methyl phosphorothioate nucleotides
  modified_base 97..99: mod_base = OTHER; note = 2-O-methyl phosphorothioate nucleotides
ggggcagctccggcgctcctgttttagagctagaaatagcaagttaaaataaggctagtccgttatcaacttgaaaaagtggcaccgagtcggtgctttt

SEQ ID NO: 46 - RNA, 100 nt, synthetic construct
  source 1..100: mol_type = other RNA
  modified_base 1..3: mod_base = OTHER; note = 2-O-methyl phosphorothioate nucleotides
  modified_base 97..99: mod_base = OTHER; note = 2-O-methyl phosphorothioate nucleotides
gaaggtggcgttgtccccttgttttagagctagaaatagcaagttaaaataaggctagtccgttatcaacttgaaaaagtggcaccgagtcggtgctttt

SEQ ID NO: 47 - RNA, 100 nt, synthetic construct
  source 1..100: mol_type = other RNA
  modified_base 1..3: mod_base = OTHER; note = 2-O-methyl phosphorothioate nucleotides
  modified_base 97..99: mod_base = OTHER; note = 2-O-methyl phosphorothioate nucleotides
gagaatcaaaatcggtgaatgttttagagctagaaatagcaagttaaaataaggctagtccgttatcaacttgaaaaagtggcaccgagtcggtgctttt

SEQ ID NO: 48 - RNA, 100 nt, synthetic construct
  source 1..100: mol_type = other RNA
  modified_base 1..3: mod_base = OTHER; note = 2-O-methyl phosphorothioate nucleotides
  modified_base 97..99: mod_base = OTHER; note = 2-O-methyl phosphorothioate nucleotides
gcgccgagaaggaagtgctcgttttagagctagaaatagcaagttaaaataaggctagtccgttatcaacttgaaaaagtggcaccgagtcggtgctttt

SEQ ID NO: 49 - RNA, 100 nt, synthetic construct
  source 1..100: mol_type = other RNA
  modified_base 1..3: mod_base = OTHER; note = 2-O-methyl phosphorothioate nucleotides
  modified_base 97..99: mod_base = OTHER; note = 2-O-methyl phosphorothioate nucleotides
gggtattattgatgctattcgttttagagctagaaatagcaagttaaaataaggctagtccgttatcaacttgaaaaagtggcaccgagtcggtgctttt

SEQ ID NO: 50 - RNA, 100 nt, synthetic construct
  source 1..100: mol_type = other RNA
  modified_base 1..3: mod_base = OTHER; note = 2-O-methyl phosphorothioate nucleotides
  modified_base 97..99: mod_base = OTHER; note = 2-O-methyl phosphorothioate nucleotides
gcacaaggctcagctgaaccgttttagagctagaaatagcaagttaaaataaggctagtccgttatcaacttgaaaaagtggcaccgagtcggtgctttt

SEQ ID NO: 51 - RNA, 100 nt, synthetic construct
  source 1..100: mol_type = other RNA
  modified_base 1..3: mod_base = OTHER; note = 2-O-methyl phosphorothioate nucleotides
  modified_base 97..99: mod_base = OTHER; note = 2-O-methyl phosphorothioate nucleotides
gtggagcgcagtggtctccggttttagagctagaaatagcaagttaaaataaggctagtccgttatcaacttgaaaaagtggcaccgagtcggtgctttt

SEQ ID NO: 52 - RNA, 100 nt, synthetic construct
  source 1..100: mol_type = other RNA
  modified_base 1..3: mod_base = OTHER; note = 2-O-methyl phosphorothioate nucleotides
  modified_base 97..99: mod_base = OTHER; note = 2-O-methyl phosphorothioate nucleotides
gagaaggtgggggggttccagttttagagctagaaatagcaagttaaaataaggctagtccgttatcaacttgaaaaagtggcaccgagtcggtgctttt

SEQ ID NO: 53 - RNA, 100 nt, synthetic construct
  source 1..100: mol_type = other RNA
  modified_base 1..3: mod_base = OTHER; note = 2-O-methyl phosphorothioate nucleotides
  modified_base 97..99: mod_base = OTHER; note = 2-O-methyl phosphorothioate nucleotides
gacaccttcttccccagcccgttttagagctagaaatagcaagttaaaataaggctagtccgttatcaacttgaaaaagtggcaccgagtcggtgctttt

SEQ ID NO: 54 - RNA, 100 nt, synthetic construct
  source 1..100: mol_type = other RNA
  modified_base 1..3: mod_base = OTHER; note = 2-O-methyl phosphorothioate nucleotides
  modified_base 97..99: mod_base = OTHER; note = 2-O-methyl phosphorothioate nucleotides
ggccgagatgtctcgctccggttttagagctagaaatagcaagttaaaataaggctagtccgttatcaacttgaaaaagtggcaccgagtcggtgctttt

SEQ ID NO: 55 - RNA, 100 nt, synthetic construct
  source 1..100: mol_type = other RNA
  modified_base 1..3: mod_base = OTHER; note = 2-O-methyl phosphorothioate nucleotides
  modified_base 97..99: mod_base = OTHER; note = 2-O-methyl phosphorothioate nucleotides
ggcagcatagtgagcccagagttttagagctagaaatagcaagttaaaataaggctagtccgttatcaacttgaaaaagtggcaccgagtcggtgctttt

SEQ ID NO: 56 - RNA, 100 nt, synthetic construct
  source 1..100: mol_type = other RNA
  modified_base 1..3: mod_base = OTHER; note = 2-O-methyl phosphorothioate nucleotides
  modified_base 97..99: mod_base = OTHER; note = 2-O-methyl phosphorothioate nucleotides
gataactacaccgaggaaatgttttagagctagaaatagcaagttaaaataaggctagtccgttatcaacttgaaaaagtggcaccgagtcggtgctttt

SEQ ID NO: 57 - RNA, 100 nt, synthetic construct
  source 1..100: mol_type = other RNA
  modified_base 1..3: mod_base = OTHER; note = 2-O-methyl phosphorothioate nucleotides
  modified_base 97..99: mod_base = OTHER; note = 2-O-methyl phosphorothioate nucleotides
gatgtgggaggctcagttccgttttagagctagaaatagcaagttaaaataaggctagtccgttatcaacttgaaaaagtggcaccgagtcggtgctttt

SEQ ID NO: 58 - RNA, 100 nt, synthetic construct
  source 1..100: mol_type = other RNA
  modified_base 1..3: mod_base = OTHER; note = 2-O-methyl phosphorothioate nucleotides
  modified_base 97..99: mod_base = OTHER; note = 2-O-methyl phosphorothioate nucleotides
ggtggatgatggtgccgtcggttttagagctagaaatagcaagttaaaataaggctagtccgttatcaacttgaaaaagtggcaccgagtcggtgctttt

SEQ ID NO: 59 - RNA, 100 nt, synthetic construct
  source 1..100: mol_type = other RNA
  modified_base 1..3: mod_base = OTHER; note = 2-O-methyl phosphorothioate nucleotides
  modified_base 97..99: mod_base = OTHER; note = 2-O-methyl phosphorothioate nucleotides
gtcgagaaaagctttgaaacgttttagagctagaaatagcaagttaaaataaggctagtccgttatcaacttgaaaaagtggcaccgagtcggtgctttt

SEQ ID NO: 60 - RNA, 100 nt, synthetic construct
  source 1..100: mol_type = other RNA
  modified_base 1..3: mod_base = OTHER; note = 2-O-methyl phosphorothioate nucleotides
  modified_base 97..99: mod_base = OTHER; note = 2-O-methyl phosphorothioate nucleotides
gctactctctctttctggccgttttagagctagaaatagcaagttaaaataaggctagtccgttatcaacttgaaaaagtggcaccgagtcggtgctttt

SEQ ID NO: 61 - RNA, 100 nt, synthetic construct
  source 1..100: mol_type = other RNA
  modified_base 1..3: mod_base = OTHER; note = 2-O-methyl phosphorothioate nucleotides
  modified_base 97..99: mod_base = OTHER; note = 2-O-methyl phosphorothioate nucleotides
gacattaaagatagtcatctgttttagagctagaaatagcaagttaaaataaggctagtccgttatcaacttgaaaaagtggcaccgagtcggtgctttt

SEQ ID NO: 62 - RNA, 100 nt, synthetic construct
  source 1..100: mol_type = other RNA
  modified_base 1..3: mod_base = OTHER; note = 2-O-methyl phosphorothioate nucleotides
  modified_base 97..99: mod_base = OTHER; note = 2-O-methyl phosphorothioate nucleotides
gccgtggcaaactggtacttgttttagagctagaaatagcaagttaaaataaggctagtccgttatcaacttgaaaaagtggcaccgagtcggtgctttt

SEQ ID NO: 63 - RNA, 100 nt, synthetic construct
  source 1..100: mol_type = other RNA
  modified_base 1..3: mod_base = OTHER; note = 2-O-methyl phosphorothioate nucleotides
  modified_base 97..99: mod_base = OTHER; note = 2-O-methyl phosphorothioate nucleotides
gggctgcaggggagctgggcgttttagagctagaaatagcaagttaaaataaggctagtccgttatcaacttgaaaaagtggcaccgagtcggtgctttt

SEQ ID NO: 64 - RNA, 100 nt, synthetic construct
  source 1..100: mol_type = other RNA
  modified_base 1..3: mod_base = OTHER; note = 2-O-methyl phosphorothioate nucleotides
  modified_base 97..99: mod_base = OTHER; note = 2-O-methyl phosphorothioate nucleotides
gggatcaggtgacccatattgttttagagctagaaatagcaagttaaaataaggctagtccgttatcaacttgaaaaagtggcaccgagtcggtgctttt

SEQ ID NO: 65 - RNA, 100 nt, synthetic construct
  source 1..100: mol_type = other RNA
  modified_base 1..3: mod_base = OTHER; note = 2-O-methyl phosphorothioate nucleotides
  modified_base 97..99: mod_base = OTHER; note = 2-O-methyl phosphorothioate nucleotides
gggtggggggagtttgctccgttttagagctagaaatagcaagttaaaataaggctagtccgttatcaacttgaaaaagtggcaccgagtcggtgctttt

SEQ ID NO: 66 - RNA, 100 nt, synthetic construct
  source 1..100: mol_type = other RNA
  modified_base 1..3: mod_base = OTHER; note = 2-O-methyl phosphorothioate nucleotides
  modified_base 97..99: mod_base = OTHER; note = 2-O-methyl phosphorothioate nucleotides
gagtagcgcgagcacagctagttttagagctagaaatagcaagttaaaataaggctagtccgttatcaacttgaaaaagtggcaccgagtcggtgctttt

SEQ ID NO: 67 - RNA, 100 nt, synthetic construct
  source 1..100: mol_type = other RNA
  modified_base 1..3: mod_base = OTHER; note = 2-O-methyl phosphorothioate nucleotides
  modified_base 97..99: mod_base = OTHER; note = 2-O-methyl phosphorothioate nucleotides
ggtgacaagtgtgatcacttgttttagagctagaaatagcaagttaaaataaggctagtccgttatcaacttgaaaaagtggcaccgagtcggtgctttt

SEQ ID NO: 68 - RNA, 100 nt, synthetic construct
  source 1..100: mol_type = other RNA
  modified_base 1..3: mod_base = OTHER; note = 2-O-methyl phosphorothioate nucleotides
  modified_base 97..99: mod_base = OTHER; note = 2-O-methyl phosphorothioate nucleotides
gtacaggctgcacctgtcaggttttagagctagaaatagcaagttaaaataaggctagtccgttatcaacttgaaaaagtggcaccgagtcggtgctttt

SEQ ID NO: 69 - RNA, 100 nt, synthetic construct
  source 1..100: mol_type = other RNA
  modified_base 1..3: mod_base = OTHER; note = 2-O-methyl phosphorothioate nucleotides
  modified_base 97..99: mod_base = OTHER; note = 2-O-methyl phosphorothioate nucleotides
gctgtttctgcagccgctttgttttagagctagaaatagcaagttaaaataaggctagtccgttatcaacttgaaaaagtggcaccgagtcggtgctttt

SEQ ID NO: 70 - RNA, 100 nt, synthetic construct
  source 1..100: mol_type = other RNA
  modified_base 1..3: mod_base = OTHER; note = 2-O-methyl phosphorothioate nucleotides
  modified_base 97..99: mod_base = OTHER; note = 2-O-methyl phosphorothioate nucleotides
gatttctatgacctgtatgggttttagagctagaaatagcaagttaaaataaggctagtccgttatcaacttgaaaaagtggcaccgagtcggtgctttt

SEQ ID NO: 71 - RNA, 100 nt, synthetic construct
  source 1..100: mol_type = other RNA
  modified_base 1..3: mod_base = OTHER; note = 2-O-methyl phosphorothioate nucleotides
  modified_base 97..99: mod_base = OTHER; note = 2-O-methyl phosphorothioate nucleotides
gaccccctccaccccgcctcgttttagagctagaaatagcaagttaaaataaggctagtccgttatcaacttgaaaaagtggcaccgagtcggtgctttt

SEQ ID NO: 72 - RNA, 100 nt, synthetic construct
  source 1..100: mol_type = other RNA
  modified_base 1..3: mod_base = OTHER; note = 2-O-methyl phosphorothioate nucleotides
  modified_base 97..99: mod_base = OTHER; note = 2-O-methyl phosphorothioate nucleotides
ggccacggagcgagacatctgttttagagctagaaatagcaagttaaaataaggctagtccgttatcaacttgaaaaagtggcaccgagtcggtgctttt

SEQ ID NO: 73 - RNA, 100 nt, synthetic construct
  source 1..100: mol_type = other RNA
  modified_base 1..3: mod_base = OTHER; note = 2-O-methyl phosphorothioate nucleotides
  modified_base 97..99: mod_base = OTHER; note = 2-O-methyl phosphorothioate nucleotides
gctgtgtttgcgtctctcccgttttagagctagaaatagcaagttaaaataaggctagtccgttatcaacttgaaaaagtggcaccgagtcggtgctttt

SEQ ID NO: 74 - RNA, 100 nt, synthetic construct
  source 1..100: mol_type = other RNA
  modified_base 1..3: mod_base = OTHER; note = 2-O-methyl phosphorothioate nucleotides
  modified_base 97..99: mod_base = OTHER; note = 2-O-methyl phosphorothioate nucleotides
gcattttcttcacggaaacagttttagagctagaaatagcaagttaaaataaggctagtccgttatcaacttgaaaaagtggcaccgagtcggtgctttt

SEQ ID NO: 75 - RNA, 100 nt, synthetic construct
  source 1..100: mol_type = other RNA
  modified_base 1..3: mod_base = OTHER; note = 2-O-methyl phosphorothioate nucleotides
  modified_base 97..99: mod_base = OTHER; note = 2-O-methyl phosphorothioate nucleotides
gctgcagaaacagcaagcccgttttagagctagaaatagcaagttaaaataaggctagtccgttatcaacttgaaaaagtggcaccgagtcggtgctttt

SEQ ID NO: 76 - RNA, 100 nt, synthetic construct
  source 1..100: mol_type = other RNA
  modified_base 1..3: mod_base = OTHER; note = 2-O-methyl phosphorothioate nucleotides
  modified_base 97..99: mod_base = OTHER; note = 2-O-methyl phosphorothioate nucleotides
ggtttcaccgagacctcagtgttttagagctagaaatagcaagttaaaataaggctagtccgttatcaacttgaaaaagtggcaccgagtcggtgctttt

SEQ ID NO: 77 - RNA, 100 nt, synthetic construct
  source 1..100: mol_type = other RNA
  modified_base 97..99: mod_base = OTHER; note = 2-O-methyl phosphorothioate nucleotides
  modified_base 1..3: mod_base = OTHER; note = 2-O-methyl phosphorothioate nucleotides
gctgaagcactgcacgccatgttttagagctagaaatagcaagttaaaataaggctagtccgttatcaacttgaaaaagtggcaccgagtcggtgctttt